European Patent Specification EP 3 941 487 B1, published February 14, 2024. Title: CD28 T CELL CULTURES, COMPOSITIONS, AND METHODS OF USING THEREOF. Applicant: Immatics US, Inc. The sequence listing filed with the application follows.

SEQUENCE LISTING (158 sequences)

SEQ ID NO: 1 - protein, 10 aa, Homo sapiens
YLYDSETKNA

SEQ ID NO: 2 - protein, 9 aa, Homo sapiens
HLMDQPLSV

SEQ ID NO: 3 - protein, 9 aa, Homo sapiens
GLLKKINSV

SEQ ID NO: 4 - protein, 9 aa, Homo sapiens
FLVDGSSAL

SEQ ID NO: 5 - protein, 10 aa, Homo sapiens
FLFDGSANLV

SEQ ID NO: 6 - protein, 9 aa, Homo sapiens
FLYKIIDEL

SEQ ID NO: 7 - protein, 11 aa, Homo sapiens
FILDSAETTTL

SEQ ID NO: 8 - protein, 9 aa, Homo sapiens
SVDVSPPKV

SEQ ID NO: 9 - protein, 8 aa, Homo sapiens
VADKIHSV

SEQ ID NO: 10 - protein, 9 aa, Homo sapiens
IVDDLTINL

SEQ ID NO: 11 - protein, 9 aa, Homo sapiens
GLLEELVTV

SEQ ID NO: 12 - protein, 10 aa, Homo sapiens
TLDGAAVNQV

SEQ ID NO: 13 - protein, 10 aa, Homo sapiens
SVLEKEIYSI

SEQ ID NO: 14 - protein, 9 aa, Homo sapiens
LLDPKTIFL

SEQ ID NO: 15 - protein, 9 aa, Homo sapiens
YTFSGDVQL

SEQ ID NO: 16 - protein, 9 aa, Homo sapiens
YLMDDFSSL

SEQ ID NO: 17 - protein, 9 aa, Homo sapiens
KVWSDVTPL

SEQ ID NO: 18 - protein, 11 aa, Homo sapiens
LLWGHPRVALA

SEQ ID NO: 19 - protein, 11 aa, Homo sapiens
KIWEELSVLEV

SEQ ID NO: 20 - protein, 9 aa, Homo sapiens
LLIPFTIFM

SEQ ID NO: 21 - protein, 9 aa, Homo sapiens
FLIENLLAA

SEQ ID NO: 22 - protein, 11 aa, Homo sapiens
LLWGHPRVALA

SEQ ID NO: 23 - protein, 9 aa, Homo sapiens
FLLEREQLL

SEQ ID NO: 24 - protein, 9 aa, Homo sapiens
SLAETIFIV

SEQ ID NO: 25 - protein, 9 aa, Homo sapiens
TLLEGISRA

SEQ ID NO: 26 - protein, 9 aa, Homo sapiens
ILQDGQFLV

SEQ ID NO: 27 - protein, 10 aa, Homo sapiens
VIFEGEPMYL

SEQ ID NO: 28 - protein, 9 aa, Homo sapiens
SLFESLEYL

SEQ ID NO: 29 - protein, 9 aa, Homo sapiens
SLLNQPKAV

SEQ ID NO: 30 - protein, 9 aa, Homo sapiens
GLAEFQENV

SEQ ID NO: 31 - protein, 9 aa, Homo sapiens
KLLAVIHEL

SEQ ID NO: 32 - protein, 9 aa, Homo sapiens
TLHDQVHLL

SEQ ID NO: 33 - protein, 11 aa, Homo sapiens
TLYNPERTITV

SEQ ID NO: 34 - protein, 9 aa, Homo sapiens
KLQEKIQEL

SEQ ID NO: 35 - protein, 10 aa, Homo sapiens
SVLEKEIYSI

SEQ ID NO: 36 - protein, 11 aa, Homo sapiens
RVIDDSLVVGV

SEQ ID NO: 37 - protein, 9 aa, Homo sapiens
VLFGELPAL

SEQ ID NO: 38 - protein, 9 aa, Homo sapiens
GLVDIMVHL

SEQ ID NO: 39 - protein, 9 aa, Homo sapiens
FLNAIETAL

SEQ ID NO: 40 - protein, 9 aa, Homo sapiens
ALLQALMEL

SEQ ID NO: 41 - protein, 9 aa, Homo sapiens
ALSSSQAEV

SEQ ID NO: 42 - protein, 11 aa, Homo sapiens
SLITGQDLLSV

SEQ ID NO: 43 - protein, 9 aa, Homo sapiens
QLIEKNWLL

SEQ ID NO: 44 - protein, 9 aa, Homo sapiens
LLDPKTIFL

SEQ ID NO: 45 - protein, 9 aa, Homo sapiens
RLHDENILL

SEQ ID NO: 46 - protein, 9 aa, Homo sapiens
YTFSGDVQL

SEQ ID NO: 47 - protein, 9 aa, Homo sapiens
GLPSATTTV

SEQ ID NO: 48 - protein, 11 aa, Homo sapiens
GLLPSAESIKL

SEQ ID NO: 49 - protein, 9 aa, Homo sapiens
KTASINQNV

SEQ ID NO: 50 - protein, 9 aa, Homo sapiens
SLLQHLIGL

SEQ ID NO: 51 - protein, 9 aa, Homo sapiens
YLMDDFSSL

SEQ ID NO: 52 - protein, 9 aa, Homo sapiens
LMYPYIYHV

SEQ ID NO: 53 - protein, 9 aa, Homo sapiens
KVWSDVTPL

SEQ ID NO: 54 - protein, 11 aa, Homo sapiens
LLWGHPRVALA

SEQ ID NO: 55 - protein, 9 aa, Homo sapiens
VLDGKVAVV

SEQ ID NO: 56 - protein, 9 aa, Homo sapiens
GLLGKVTSV

SEQ ID NO: 57 - protein, 9 aa, Homo sapiens
KMISAIPTL

SEQ ID NO: 58 - protein, 11 aa, Homo sapiens
GLLETTGLLAT

SEQ ID NO: 59 - protein, 9 aa, Homo sapiens
TLNTLDINL

SEQ ID NO: 60 - protein, 9 aa, Homo sapiens
VIIKGLEEI

SEQ ID NO: 61 - protein, 9 aa, Homo sapiens
YLEDGFAYV

SEQ ID NO: 62 - protein, 11 aa, Homo sapiens
KIWEELSVLEV

SEQ ID NO: 63 - protein, 9 aa, Homo sapiens
LLIPFTIFM

SEQ ID NO: 64 - protein, 10 aa, Homo sapiens
ISLDEVAVSL

SEQ ID NO: 65 - protein, 10 aa, Homo sapiens
KISDFGLATV

SEQ ID NO: 66 - protein, 11 aa, Homo sapiens
KLIGNIHGNEV

SEQ ID NO: 67 - protein, 9 aa, Homo sapiens
ILLSVLHQL

SEQ ID NO: 68 - protein, 9 aa, Homo sapiens
LDSEALLTL

SEQ ID NO: 69 - protein, 13 aa, Homo sapiens
VLQENSSDYQSNL

SEQ ID NO: 70 - protein, 11 aa, Homo sapiens
HLLGEGAFAQV

SEQ ID NO: 71 - protein, 9 aa, Homo sapiens
SLVENIHVL

SEQ ID NO: 72 - protein, 9 aa, Homo sapiens
YTFSGDVQL

SEQ ID NO: 73 - protein, 9 aa, Homo sapiens
SLSEKSPEV

SEQ ID NO: 74 - protein, 10 aa, Homo sapiens
AMFPDTIPRV

SEQ ID NO: 75 - protein, 9 aa, Homo sapiens
FLIENLLAA

SEQ ID NO: 76 - protein, 9 aa, Homo sapiens
FTAEFLEKV

SEQ ID NO: 77 - protein, 9 aa, Homo sapiens
ALYGNVQQV

SEQ ID NO: 78 - protein, 9 aa, Homo sapiens
LFQSRIAGV

SEQ ID NO: 79 - protein, 11 aa, Homo sapiens
ILAEEPIYIRV

SEQ ID NO: 80 - protein, 9 aa, Homo sapiens
FLLEREQLL

SEQ ID NO: 81 - protein, 10 aa, Homo sapiens
LLLPLELSLA

SEQ ID NO: 82 - protein, 9 aa, Homo sapiens
SLAETIFIV

SEQ ID NO: 83 - protein, 11 aa, Homo sapiens
AILNVDEKNQV

SEQ ID NO: 84 - protein, 9 aa, Homo sapiens
RLFEEVLGV

SEQ ID NO: 85 - protein, 9 aa, Homo sapiens
YLDEVAFML

SEQ ID NO: 86 - protein, 11 aa, Homo sapiens
KLIDEDEPLFL

SEQ ID NO: 87 - protein, 9 aa, Homo sapiens
KLFEKSTGL

SEQ ID NO: 88 - protein, 11 aa, Homo sapiens
SLLEVNEASSV

SEQ ID NO: 89 - protein, 10 aa, Homo sapiens
GVYDGREHTV

SEQ ID NO: 90 - protein, 10 aa, Homo sapiens
GLYPVTLVGV

SEQ ID NO: 91 - protein, 9 aa, Homo sapiens
ALLSSVAEA

SEQ ID NO: 92 - protein, 9 aa, Homo sapiens
TLLEGISRA

SEQ ID NO: 93 - protein, 9 aa, Homo sapiens
SLIEESEEL

SEQ ID NO: 94 - protein, 9 aa, Homo sapiens
ALYVQAPTV

SEQ ID NO: 95 - protein, 10 aa, Homo sapiens
KLIYKDLVSV

SEQ ID NO: 96 - protein, 9 aa, Homo sapiens
ILQDGQFLV

SEQ ID NO: 97 - protein, 9 aa, Homo sapiens
SLLDYEVSI

SEQ ID NO: 98 - protein, 9 aa, Homo sapiens
LLGDSSFFL

SEQ ID NO: 99 - protein, 10 aa, Homo sapiens
VIFEGEPMYL

SEQ ID NO: 100 - protein, 9 aa, Homo sapiens
ALSYILPYL

SEQ ID NO: 101 - protein, 9 aa, Homo sapiens
FLFVDPELV

SEQ ID NO: 102 - protein, 11 aa, Homo sapiens
SEWGSPHAAVP

SEQ ID NO: 103 - protein, 9 aa, Homo sapiens
ALSELERVL

SEQ ID NO: 104 - protein, 9 aa, Homo sapiens
SLFESLEYL

SEQ ID NO: 105 - protein, 9 aa, Homo sapiens
KVLEYVIKV

SEQ ID NO: 106 - protein, 10 aa, Homo sapiens
VLLNEILEQV

SEQ ID NO: 107 - protein, 9 aa, Homo sapiens
SLLNQPKAV

SEQ ID NO: 108 - protein, 9 aa, Homo sapiens
KMSELQTYV

SEQ ID NO: 109 - protein, 11 aa, Homo sapiens
ALLEQTGDMSL

SEQ ID NO: 110 - protein, 11 aa, Homo sapiens
VIIKGLEEITV

SEQ ID NO: 111 - protein, 9 aa, Homo sapiens
KQFEGTVEI

SEQ ID NO: 112 - protein, 9 aa, Homo sapiens
KLQEEIPVL

SEQ ID NO: 113 - protein, 9 aa, Homo sapiens
GLAEFQENV

SEQ ID NO: 114 - protein, 9 aa, Homo sapiens
NVAEIVIHI

SEQ ID NO: 115 - protein, 9 aa, Homo sapiens
ALAGIVTNV

SEQ ID NO: 116 - protein, 12 aa, Homo sapiens
NLLIDDKGTIKL

SEQ ID NO: 117 - protein, 10 aa, Homo sapiens
VLMQDSRLYL

SEQ ID NO: 118 - protein, 9 aa, Homo sapiens
KVLEHVVRV

SEQ ID NO: 119 - protein, 9 aa, Homo sapiens
LLWGNLPEI

SEQ ID NO: 120 - protein, 9 aa, Homo sapiens
SLMEKNQSL

SEQ ID NO: 121 - protein, 9 aa, Homo sapiens
KLLAVIHEL

SEQ ID NO: 122 - protein, 10 aa, Homo sapiens
ALGDKFLLRV

SEQ ID NO: 123 - protein, 11 aa, Homo sapiens
FLMKNSDLYGA

SEQ ID NO: 124 - protein, 10 aa, Homo sapiens
KLIDHQGLYL

SEQ ID NO: 125 - protein, 12 aa, Homo sapiens
GPGIFPPPPPQP

SEQ ID NO: 126 - protein, 9 aa, Homo sapiens
ALNESLVEC

SEQ ID NO: 127 - protein, 9 aa, Homo sapiens
GLAALAVHL

SEQ ID NO: 128 - protein, 9 aa, Homo sapiens
LLLEAVWHL

SEQ ID NO: 129 - protein, 9 aa, Homo sapiens
SIIEYLPTL

SEQ ID NO: 130 - protein, 9 aa, Homo sapiens
TLHDQVHLL

SEQ ID NO: 131 - protein, 9 aa, Homo sapiens
SLLMWITQC

SEQ ID NO: 132 - protein, 11 aa, Homo sapiens
FLLDKPQDLSI

SEQ ID NO: 133 - protein, 10 aa, Homo sapiens
YLLDMPLWYL

SEQ ID NO: 134 - protein, 9 aa, Homo sapiens
GLLDCPIFL

SEQ ID NO: 135 - protein, 9 aa, Homo sapiens
VLIEYNFSI

SEQ ID NO: 136 - protein, 11 aa, Homo sapiens
TLYNPERTITV

SEQ ID NO: 137 - protein, 9 aa, Homo sapiens
AVPPPPSSV

SEQ ID NO: 138 - protein, 9 aa, Homo sapiens
KLQEELNKV

SEQ ID NO: 139 - protein, 11 aa, Homo sapiens
KLMDPGSLPPL

SEQ ID NO: 140 - protein, 9 aa, Homo sapiens
ALIVSLPYL

SEQ ID NO: 141 - protein, 9 aa, Homo sapiens
FLLDGSANV

SEQ ID NO: 142 - protein, 10 aa, Homo sapiens
ALDPSGNQLI

SEQ ID NO: 143 - protein, 9 aa, Homo sapiens
ILIKHLVKV

SEQ ID NO: 144 - protein, 9 aa, Homo sapiens
VLLDTILQL

SEQ ID NO: 145 - protein, 9 aa, Homo sapiens
HLIAEIHTA

SEQ ID NO: 146 - protein, 9 aa, Homo sapiens
SMNGGVFAV

SEQ ID NO: 147 - protein, 9 aa, Homo sapiens
MLAEKLLQA

SEQ ID NO: 148 - protein, 9 aa, Homo sapiens
YMLDIFHEV

SEQ ID NO: 149 - protein, 11 aa, Homo sapiens
ALWLPTDSATV

SEQ ID NO: 150 - protein, 9 aa, Homo sapiens
GLASRILDA

SEQ ID NO: 151 - protein, 9 aa, Homo sapiens
ALSVLRLAL

SEQ ID NO: 152 - protein, 9 aa, Homo sapiens
SYVKVLHHL

SEQ ID NO: 153 - protein, 9 aa, Homo sapiens
VYLPKIPSW

SEQ ID NO: 154 - protein, 9 aa, Homo sapiens
NYEDHFPLL

SEQ ID NO: 155 - protein, 9 aa, Homo sapiens
VYIAELEKI

SEQ ID NO: 156 - protein, 12 aa, Homo sapiens
VHFEDTGKTLLF

SEQ ID NO: 157 - protein, 9 aa, Homo sapiens
VLSPFILTL

SEQ ID NO: 158 - protein, 9 aa, Homo sapiens
HLLEGSVGV